European Patent Application EP 4 177 262 A1, published May 10, 2023. Title: Novel proteins specific for CD137. Applicant: Pieris Pharmaceuticals GmbH. The sequence listing filed with the application follows.

SEQUENCE LISTING (39 sequences)

SEQ ID NO: 1 - protein, 156 aa, synthetic construct
  REGION 1..156: note = wildtype human Tlc
HHLLASDEEIQDVSGTWYLKAMTVDREFPEMNLESVTPMTLTTLEGGNLEAKVTMLISGRCQEVKAVLEKTDEPGKYTADGGKHVAYIIRSHVKDHYIFYCEGELHGKPVRGVKLVGRDPKNNLEALEDFEKAAGARGLSTESILIPRQSETCSPG

SEQ ID NO: 2 - protein, 178 aa, synthetic construct
  REGION 1..178: note = wildtype hNGAL
QDSTSDLIPAPPLSKVPLQQNFQDNQFQGKWYVVGLAGNAILREDKDPQKMYATIYELKEDKSYNVTSVLFRKKKCDYWIRTFVPGCQPGEFTLGNIKSYPGLTSYLVRVVSTNYNQHAMVFFKKVSQNREYFKITLYGRTKELTSELKENFIRFSKSLGLPENHIVFPVPIDQCIDG

SEQ ID NO: 3 - protein, 152 aa, synthetic construct
  REGION 1..152: note = negative control
ASDEEIQDVSGTWYLKAMTVDRECPEMNLESVTPMTLTTLEGGNLEAKVTMLISGRSQEVKAVLEKTDEPGKYTADGGKHVAYIIRSHVKDHYIFYSEGECHGKPVPGVWLVGRDPKNNLEALEDFEKAAGARGLSTESILIPRQSETSSPG

SEQ ID NO: 4 - protein, 178 aa, synthetic construct
  REGION 1..178: note = negative control
QDSTSDLIPAPPLSKVPLQQNFQDNQFHGKWYVVGLAGNAILREDKDPQKMYATIYELKEDKSYNVTSVLFRKKKCDYWIRTFVPGSQPGEFTLGNIKSYPGLTSYLVRVVSTNYNQHAMVFFKKVSQNREYFKITLYGRTKELTSELKENFIRFSKSLGLPENHIVFPVPIDQCIDG

SEQ ID NO: 5 - protein, 152 aa, synthetic construct
  REGION 1..152: note = lipocalin mutein
ASDEEIQDVSGTWYLKAMTVDEGCRPWNIFSVTPMTLTTLEGGNLEAKVTMAIDGPAQEVKAVLEKTDEPGKYTADGGKHVAYIIRSHVKDHYIFYSEGVCDGSPVPGVWLVGRDPKNNLEALEDFEKAAGARGLSTESILIPRQSETSSPG

SEQ ID NO: 6 - protein, 152 aa, synthetic construct
  REGION 1..152: note = lipocalin mutein
TSDEEIQDVSGTWYLKAMTVDEGCRPWNIFSVTPMTLTTLEGGNLEAKVTMAIDGPAQEVRAVLEKTDEPGKYTADGGKHDAYIIRSHVKDHYIFYSEGVCDGSPVPGVWLVGRDPENNLEALEDFEKTAGARGLSTESILIPRQSETSSPG

SEQ ID NO: 7 - protein, 152 aa, synthetic construct
  REGION 1..152: note = lipocalin mutein
ASDEEIQDVSGTWYLKAMTVDEGCRPWNIFSVTPMTLTTLEGGNLEAKVTMAIDGPAQEVNAVLEKTDEPGKYTADGGKHVAYIIRSHVRDHYIFYSEGVCDGSPVPGVWLVGRDPENNLEALEDFEKTAGARGLSTESILIPRQSETSSPG

SEQ ID NO: 8 - protein, 152 aa, synthetic construct
  REGION 1..152: note = lipocalin mutein
VSDEEIQDVSGTWYLKAMTVDEGCRPWNIFSVTPMTLTTLEGGNLEAKVTMAIDGPAQEVRAVLEKTDEPGKYTADGGKHVAYIIRSHVEDHYIFYSEGVCDGSPVPGVWLVGRDPENNLEALEDFEKTAGARGLSTESILIPRQSETSSPG

SEQ ID NO: 9 - protein, 152 aa, synthetic construct
  REGION 1..152: note = lipocalin mutein
ASDEEIQDVSGTWYLKAMTVDEGCRPWNIFSVTPMTLSTLEGGNLEAKVTMAIDGPAQEVKAVLEKTDEPGKYTADGGKHVAYIIRSHVKDHYIFYSEGVCDGSPVPGVWLVGRDPKNNLEALEDFEKAAGARGLSTESILIPRQIETSSPG

SEQ ID NO: 10 - protein, 152 aa, synthetic construct
  REGION 1..152: note = lipocalin mutein
ASDEEIQDVSGTWYLKAMTVDEGCRPWNIFSVTPMTLTTLEGGNLEAEVTMAIDGPAQEVKAVLEKADEPGKYTADGGKHVAYIIRSHVKDHYIFYSEGVCDGSPVPGVWLVGRDPKNNLEALEDFEKTAGARGLSTESILIPSQIETSSPG

SEQ ID NO: 11 - protein, 152 aa, synthetic construct
  REGION 1..152: note = lipocalin mutein
TSDEEIQDVSGTWYLKAMTVDEGCRPWNIFSVTPMTLTTLEDGNLEAKVTMAIDGPAQEVKAVLEKADEPGKYTADGGKHVAYIIRSHVKDHYIFYSEGVCDGSPVPGVWLVGRDPKNNLEALEDFEKAAGARGLSTESILIPRQIETSSPG

SEQ ID NO: 12 - protein, 178 aa, synthetic construct
  REGION 1..178: note = lipocalin mutein
QDSTSDLIPAPPLSKVPLQQNFQDNQFHGKWYVVGQAGNIKLREDKDPNKMMATIYELKEDKSYNVTGVTFDDKKCTYAISTFVPGSQPGEFTLGKIKSFPGHTSSLVRVVSTNYNQHAMVFFKFVFQNREEFYITLYGRTKELTSELKENFIRFSKSLGLPENHIVFPVPIDQCIDG

SEQ ID NO: 13 - protein, 178 aa, synthetic construct
  REGION 1..178: note = lipocalin mutein
QDSTSDLIPAPPLSKVPLQQNFQDNQFHGKWYVVGQAGNIRLREDKDPIKMMATIYELKEDKSYDVTMVKFDDKKCMYDIWTFVPGSQPGEFTLGKIKSFPGHTSSLVRVVSTNYNQHAMVFFKFVFQNREEFYITLYGRTKELTSELKENFIRFSKSLGLPENHIVFPVPIDQCIDG

SEQ ID NO: 14 - protein, 178 aa, synthetic construct
  REGION 1..178: note = lipocalin mutein
QDSTSDLIPAPPLSKVPLQQNFQDNQFHGKWYVVGQAGNIRLREDKDPNKMMATIYELKEDKSYDVTAVAFDDKKCTYDIWTFVPGSQPGEFTLGKIKSFPGHTSSLVRVVSTNYNQHAMVFFKFVFQNREEFYITLYGRTKELTSELKENFIRFSKSLGLPENHIVFPVPIDQCIDG

SEQ ID NO: 15 - protein, 178 aa, synthetic construct
  REGION 1..178: note = lipocalin muein
QDSTSDLIPAPPLSKVPLQQNFQDNQFHGKWYVVGQAGNIKLREDKDPNKMMATIYELKEDKSYDVTAVAFDDKKCTYDIWTFVPGSQPGEFTLGKIKSFPGHTSSLVRVVSTNYNQHAMVFFKFVFQNREEFYITLYGRTKELTSELKENFIRFSKSLGLPENHIVFPVPIDQCIDG

SEQ ID NO: 16 - protein, 175 aa, synthetic construct
  REGION 1..175: note = lipocalin mutein
QDSTSDLIPAPPLSKVPLQQNFQDNQFHGKWYVVGQAGNIKLREDSKMMATIYELKEDKSYDVTGVSFDDKKCTYAIMTFVPGSQPGEFTLGKIKSFPGHTSSLVRVVSTNYNQHAMVFFKFVFQNREEFYITLYGRTKELTSELKENFIRFSKSLGLPENHIVFPVPIDQCIDG

SEQ ID NO: 17 - protein, 178 aa, synthetic construct
  REGION 1..178: note = lipocalin mutein
QDSTSDLIPAPPLSKVPLQQNFQDNQFHGKWYVVGQAGNIKLREDKDPVKMMATIYELKEDKSYDVTGVTFDDKKCRYDISTFVPGSQPGEFTFGKIKSFPGHTSSLVRVVSTNYNQHAMVFFKFVFQNREEFYITLYGRTKELTSELKENFIRFSKSLGLPENHIVFPVPIDQCIDG

SEQ ID NO: 18 - protein, 178 aa, synthetic construct
  REGION 1..178: note = lipocalin mutein
QDSTSDLIPAPPLSKVPLQQNFQDNQFHGKWYVVGQAGNIRLREDKDPHKMMATIYELKEDKSYDVTGVTFDDKKCTYAISTFVPGSQPGEFTLGKIKSFPGHTSSLVRVVSTNYNQHAMVFFKFVFQNREEFYITLYGRTKELTSELKENFIRFSKSLGLPENHIVFPVPIDQCIDG

SEQ ID NO: 19 - protein, 178 aa, synthetic construct
  REGION 1..178: note = lipocalin mutein
QDSTSDLIPAPPLSKVPLQQNFQDNQFHGKWYVVGQAGNIKLREDKDPNKMMATIYELKEDKSYDVTGVTFDDKKCTYAISTLVPGSQPGEFTFGKIKSFPGHTSSLVRVVSTNYNQHAMVFFKFVFQNREEFYITLYGRTKELTSELKENFIRFSKSLGLPENHIVFPVPIDQCIDG

SEQ ID NO: 20 - protein, 178 aa, synthetic construct
  REGION 1..178: note = lipocalin mutein
QDSTSDLIPAPPLSKVPLQQNFQDNQFHGKWYVVGQAGNIRLREDKDPSKMMATIYELKEDKSYDVTAVTFDDKKCNYAISTFVPGSQPGEFTLGKIKSFPGHTSSLVRVVSTNYNQHAMVFFKFVFQNREEFYITLYGRTKELTSELKENFIRFSKSLGLPENHIVFPVPIDQCIDG

SEQ ID NO: 21 - protein, 10 aa, synthetic construct
  REGION 1..10: note = C-terminal tag 1
SAWSHPQFEK

SEQ ID NO: 22 - protein, 11 aa, synthetic construct
  REGION 1..11: note = C-terminal tag 2
PSAWSHPQFEK

SEQ ID NO: 23 - protein, 8 aa, synthetic construct
  REGION 1..8: note = Strep-tag
WSHPQFEK

SEQ ID NO: 24 - DNA, 456 bp, synthetic construct
  misc_feature 1..456: note = lipocalin mutein
  source 1..456: mol_type = other DNA
gcctcagacgaggagattcaggatgtgtcagggacgtggtatctgaaggccatgacggtggatgaggggtgtcgtccttggaatatattttcagttacgccaatgactctgactacccttgaaggcggcaatctggaggctaaggtcaccatggcaatagatgggccggcacaggaggtgaaagcagtgttagagaagacagatgaaccgggtaaatatacggccgatggcggtaaacatgttgcctatatcattcgcagccatgtgaaagatcattacatcttttatagcgagggcgtgtgcgatgggtctcctgttccaggggtgtggctcgtgggcagagaccccaagaacaacctggaagccttggaggactttgagaaagccgcaggagcccgcggactcagcacggagagcatcctcatccccaggcagagcgaaaccagctctccaggg

SEQ ID NO: 25 - DNA, 459 bp, synthetic construct
  misc_feature 1..459: note = lipocalin mutein
  source 1..459: mol_type = other DNA
acctcagacgaggagattcaggatgtgtcagggacgtggtatctgaaggcgatgacggtggatgaggggtgtcgtccttggaatatattttcagttacgccaatgactctgactacccttgaaggcggcaatctggaggctaaggtcaccatggcaatagatgggccggcacaggaggtgagagcagtgttagagaagacagatgaaccgggtaaatatacggccgacggcggtaaacatgatgcctatatcattcgcagccatgtgaaagatcattacatcttttatagcgagggcgtgtgcgatgggtctcctgttccgggggtgtggctcgtgggcagagaccccgagaacaacctggaagccttggaggactttgagaaaaccgcaggagcccgcggactcagcacggagagcatcctcatccccaggcagagcgaaaccagctctccagggcca

SEQ ID NO: 26 - DNA, 456 bp, synthetic construct
  misc_feature 1..456: note = lipocalin mutein
  source 1..456: mol_type = other DNA
gcctcagacgaggagattcaggatgtgtcagggacgtggtatctgaaggcgatgacggtggatgaggggtgtcgtccttggaatatattttcagttacgccaatgactctgactacccttgaaggcggcaatctggaggctaaggtcaccatggcaatagatgggccggcacaggaggtgaacgcagtgttagagaagacagatgaaccgggtaaatatacggccgatggcggtaaacatgttgcctatatcattcgcagccatgtgagagatcattacatcttttatagcgagggcgtgtgcgatgggtctcctgttccgggggtgtggctcgtgggcagggaccccgagaacaacctggaagccttggaggactttgagaaaaccgcaggagcccgcggactcagcacggagagcattctcattcccaggcagagcgaaaccagctctccaggg

SEQ ID NO: 27 - DNA, 459 bp, synthetic construct
  misc_feature 1..459: note = lipocalin mutein
  source 1..459: mol_type = other DNA
gtctcagacgaggagattcaggatgtgtcagggacgtggtatctgaaggcgatgacggtggatgaggggtgtcgtccttggaatatattttcagttacgccaatgactctgactacccttgaaggcggcaatctggaggctaaggtcaccatggcaatagatgggccggcacaggaggtgagagcagtgttagagaagacagatgaaccgggtaaatatacggccgatggcggtaaacatgttgcctatatcattcgcagccatgtggaagatcattacatcttttatagcgagggcgtgtgcgatgggtctcctgttccgggggtgtggctcgtgggcagagaccccgagaacaacctggaagccttggaggactttgagaaaaccgcaggagcccgcggactcagcacggagagcatcctcatccccaggcagagcgaaaccagctctccagggcca

SEQ ID NO: 28 - DNA, 459 bp, synthetic construct
  misc_feature 1..459: note = lipocalin mutein
  source 1..459: mol_type = other DNA
gcctcagacgaggagattcaggatgtgtcagggacgtggtatctgaaggcgatgacggtggatgaggggtgtcgtccttggaatatattttcagttacgccaatgactctgtctacccttgaaggcggcaatctggaggctaaggtcaccatggcaatagatgggccggcacaggaggtgaaagcagtgttagagaagacagatgaaccgggtaaatatacggccgatggcggtaaacatgttgcctatatcattcgcagccatgtgaaagatcattacatcttttatagcgagggcgtgtgcgatgggtctcctgttccgggggtgtggctcgtgggcagagaccccaagaacaacctggaagccttggaggactttgagaaagccgcaggagcccgcggactcagcacggagagcatcctcatccccaggcagatcgaaaccagctctccagggcca

SEQ ID NO: 29 - DNA, 459 bp, synthetic construct
  misc_feature 1..459: note = lipocalin mutein
  source 1..459: mol_type = other DNA
gcctcagacgaggagattcaggatgtgtcagggacgtggtatctgaaggcgatgacggtggatgaggggtgtcgtccttggaatatattttcagttacgccaatgactctgactacccttgaaggcggcaatctggaggctgaggtcaccatggcaatagatgggccggcacaggaggtgaaagcagtgttagagaaggcagatgaaccgggtaaatatacggccgatggcggtaaacatgttgcctatatcattcgcagccatgtgaaagatcattacatcttttatagcgagggcgtgtgcgatgggtctcctgttccgggggtgtggctcgtgggcagagaccccaagaacaacctggaagccttggaggactttgagaaaaccgcaggagcccgcggactcagcacggagagcatcctcatccccagtcagatcgaaaccagctctccagggcca

SEQ ID NO: 30 - DNA, 459 bp, synthetic construct
  misc_feature 1..459: note = lipocalin mutein
  source 1..459: mol_type = other DNA
acctcagacgaggagattcaggatgtgtcagggacgtggtatctgaaggcgatgacggtggatgaggggtgtcgtccttggaatatattttcagttacgccaatgactctgactacccttgaagacggcaatctggaggctaaggtcaccatggcaatagatgggccggcacaggaggtgaaagcagtgttagagaaggcagatgaaccgggtaaatatacggccgatggcggtaaacatgttgcctatatcattcgcagccatgtgaaagatcattacatcttttatagcgagggcgtgtgcgatgggtctcctgttccgggggtgtggctcgtgggcagagaccccaagaacaacctggaagccttggaggactttgagaaagccgcaggagcccgcggactcagcacggagagcatcctcatccccaggcagatcgaaaccagctctccagggcca

SEQ ID NO: 31 - DNA, 534 bp, synthetic construct
  misc_feature 1..534: note = lipocalin mutein
  source 1..534: mol_type = other DNA
caggactccacctcagacctgatcccagccccacctctgagcaaggtccctctgcagcagaacttccaggacaaccaattccatgggaagtggtatgtggtaggtcaggcagggaatatcaaactcagagaagacaaagacccgaacaagatgatggccaccatctatgagctgaaagaagacaagagctacaatgtcaccggtgtcacttttgacgacaagaagtgtacttacgctatctctacttttgttccaggttcccagccaggcgagttcacgctgggcaaaattaagagtttccctggacatacgagttctctcgtccgagtggtgagcaccaactacaaccagcatgctatggtgttcttcaagttcgttttccaaaacagggaggaattctacatcaccctctacgggagaaccaaggagctgacttcggaactaaaggagaacttcatccgcttctccaaatctctgggcctccctgaaaaccacatcgtcttccctgtcccaatcgaccagtgtatcgacggc

SEQ ID NO: 32 - DNA, 534 bp, synthetic construct
  misc_feature 1..534: note = lipocalin mutein
  source 1..534: mol_type = other DNA
caggactccacctcagacctgatcccagccccacctctgagcaaggtccctctgcagcagaacttccaggacaaccaattccatgggaaatggtacgttgtcgggcaggccggaaatattaggctgcgtgaggataaggatccgattaaaatgatggcgaccatttacgagttgaaagaagataaatcatatgacgtcaccatggtgaagtttgatgataagaaatgcatgtacgatatttggacctttgtgccggggagccagccgggcgagtttactttaggcaagattaaaagttttccgggccatacatcatcgttggtccgcgtcgtgagcaccaactacaaccagcatgccatggtgttcttcaagtttgtgtttcagaaccgcgaggagttttatatcacactgtacgggcgcacgaaagaactgacaagcgagctgaaggaaaattttatccgcttttccaaatctctgggcctccctgaaaaccacatcgtcttccctgtcccaatcgaccagtgtatcgacggc

SEQ ID NO: 33 - DNA, 534 bp, synthetic construct
  misc_feature 1..534: note = lipocalin mutein
  source 1..534: mol_type = other DNA
caggactccacctcagacctgatcccagccccacctctgagcaaggtccctctgcagcagaacttccaggacaaccaattccatgggaaatggtacgttgtcgggcaggccggaaatattaggctgcgtgaggataaggatccgaataaaatgatggcgaccatttacgagttgaaagaagataaatcatatgacgtcaccgcggtggcgtttgatgataagaaatgcacgtacgatatttggacctttgtgccggggagccagccgggcgagtttactttaggcaagattaaaagttttccgggccatacatcatcgttggtccgcgtcgtgagcaccaactacaaccagcatgccatggtgttcttcaagtttgtgtttcagaaccgcgaggagttttatatcacactgtacgggcgcacgaaagaactgacaagcgagctgaaggaaaattttatccgcttttccaaatctctgggcctccctgaaaaccacatcgtcttccctgtcccaatcgaccagtgtatcgacggc

SEQ ID NO: 34 - DNA, 534 bp, synthetic construct
  misc_feature 1..534: note = lipocalin mutein
  source 1..534: mol_type = other DNA
caggactccacctcagacctgatcccagccccacctctgagcaaggtccctctgcagcagaacttccaggacaaccaattccatgggaaatggtacgttgtcgggcaggccggaaatattaagctgcgtgaggataaggatccgaataaaatgatggcgaccatttacgagttgaaagaagataaatcatatgacgtcaccgcggtggcgtttgatgataagaaatgcacgtacgatatttggacctttgtgccggggagccagccgggcgagtttactttaggcaagattaaaagttttccgggccatacatcatctttggtccgcgtcgtgagcaccaactacaaccagcatgccatggtgttcttcaagtttgtgtttcagaaccgcgaggagttttatatcacactgtacgggcgcacgaaagaactgacaagcgagctgaaggaaaattttatccgcttttccaaatctctgggcctccctgaaaaccacatcgtcttccctgtcccaatcgaccagtgtatcgacggc

SEQ ID NO: 35 - DNA, 525 bp, synthetic construct
  misc_feature 1..525: note = lipocalin mutein
  source 1..525: mol_type = other DNA
caggactccacctcagacctgatcccagccccacctctgagcaaggtccctctgcagcagaacttccaggacaaccaattccatgggaaatggtacgttgtcgggcaggccggaaatattaagctgcgtgaggatagtaaaatgatggcgaccatttacgagttgaaagaagataaatcatatgacgtcaccggtgtgagttttgatgataagaaatgcacgtacgctattatgacctttgtgccggggagccagccgggcgagtttactttaggcaagattaaaagttttccgggccatacatcatcgttggtccgcgtcgtgagcaccaactacaaccagcatgccatggtgttcttcaagtttgtgtttcagaaccgcgaggagttttatatcacactgtacgggcgcacgaaagaactgacaagcgagctgaaggaaaattttatccgcttttccaaatctctgggcctccctgaaaaccacatcgtcttccctgtcccaatcgaccagtgtatcgacggc

SEQ ID NO: 36 - DNA, 534 bp, synthetic construct
  misc_feature 1..534: note = lipocalin mutein
  source 1..534: mol_type = other DNA
caggactccacctcagacctgatcccagccccacctctgagcaaggtccctctgcagcagaacttccaggacaaccaattccatgggaaatggtacgttgtcgggcaggccggaaatattaagctgcgtgaggataaggatccggttaaaatgatggcgaccatttacgagttgaaagaagataaatcatatgacgtcaccggggtgacgtttgatgataagaaatgcaggtacgatatttcgacctttgtgccggggagccagccgggcgagtttacttttggcaagattaaaagttttccgggccatacatcatcgttggtccgcgtcgtgagcaccaactacaaccagcatgccatggtgttcttcaagtttgtgtttcagaaccgcgaggagttttatatcacactgtacgggcgcacgaaagaactgacaagcgagctgaaggaaaattttatccgcttttccaaatctctgggcctccctgaaaaccacatcgtcttccctgtcccaatcgaccagtgtatcgacggc

SEQ ID NO: 37 - DNA, 534 bp, synthetic construct
  misc_feature 1..534: note = lipocalin mutein
  source 1..534: mol_type = other DNA
caggactccacctcagacctgatcccagccccacctctgagcaaggtccctctgcagcagaacttccaggacaaccaattccatgggaaatggtacgttgtcgggcaggccggaaatattaggctgcgtgaggataaggatccgcataaaatgatggcgaccatttacgagttgaaagaagataaatcatatgacgtcaccggggtgacttttgatgataagaaatgcacgtacgctatttcgacctttgtgccggggagccagccgggcgagtttactttaggcaagattaaaagttttccgggccatacatcatctttggtccgcgtcgtgagcaccaactacaaccagcatgccatggtgttcttcaagtttgtgtttcagaaccgcgaggagttttatatcacactgtacgggcgcacgaaagaactgacaagcgagctgaaggaaaattttatccgcttttccaaatctctgggcctccctgaaaaccacatcgtcttccctgtcccaatcgaccagtgtatcgacggc

SEQ ID NO: 38 - DNA, 534 bp, synthetic construct
  misc_feature 1..534: note = lipocalin mutein
  source 1..534: mol_type = other DNA
caggactccacctcagacctgatcccagccccacctctgagcaaggtccctctgcagcagaacttccaggacaaccaattccatgggaaatggtacgttgtcgggcaggccggaaatattaagctgcgtgaggataaggatccgaataaaatgatggcgaccatttacgagttgaaagaagataaatcatatgacgtcaccggggtgacttttgatgataagaaatgcacgtacgctatttctacccttgtgccggggagccagccgggcgagtttacttttggcaagattaaaagttttccgggccatacatcatcgttggtccgcgtcgtgagcaccaactacaaccagcatgccatggtgttcttcaagtttgtgtttcagaaccgcgaggagttttatatcacactgtacgggcgcacgaaagaactgacaagcgagctgaaggaaaattttatccgcttttccaaatctctgggcctccctgaaaaccacatcgtcttccctgtcccaatcgaccagtgtatcgacggc

SEQ ID NO: 39 - DNA, 534 bp, synthetic construct
  misc_feature 1..534: note = lipocalin mutein
  source 1..534: mol_type = other DNA
caggactccacctcagacctgatcccagccccacctctgagcaaggtccctctgcagcagaacttccaggacaaccaattccatgggaaatggtacgttgtcgggcaggccggaaatattaggctgcgtgaggataaggatccgtctaaaatgatggcgaccatttacgagttgaaagaagataaatcatatgacgtcaccgctgtgacgtttgatgataagaaatgcaattacgctatttctacctttgtgccggggagccagccgggcgagtttactttaggcaagattaaaagttttccgggccatacatcatcgttggtccgcgtcgtgagcaccaactacaaccagcatgccatggtgttcttcaagtttgtgtttcagaaccgcgaggagttttatatcacactgtacgggcgcacgaaagaactgacaagcgagctgaaggaaaattttatccgcttttccaaatctctgggcctccctgaaaaccacatcgtcttccctgtcccaatcgaccagtgtatcgacggc